European Patent Specification EP 3 901 164 B1, published November 20, 2024. Title: Gluten-Related Disorders. Applicant: H.J. Heinz Company. The sequence listing filed with the application follows.

SEQUENCE LISTING (10 sequences)

SEQ ID NO: 1 - protein, 13 aa, Triticum aestivum
LGQQQPFPPQQPY

SEQ ID NO: 2 - protein, 12 aa, Triticum aestivum
QLQPFPQPQLPY

SEQ ID NO: 3 - protein, 19 aa, Triticum aestivum
LGQQQPFPPQQPYPQPQPF

SEQ ID NO: 4 - protein, 33 aa, Triticum aestivum
LQLQPFPQPQLPYPQPQLPYPQPQLPYPQPQPF

SEQ ID NO: 5 - protein, 10 aa, Triticum aestivum
PQQPFPSQLP

SEQ ID NO: 6 - protein, 14 aa, Triticum aestivum
QPQLPYPQPQLPYP

SEQ ID NO: 7 - protein, 290 aa, Triticum aestivum
MVRVPVPQLQPQNPSQQQPQEQVPLVQQQQFPGQQQPFPPQQPYPQPQPFPSQQPYLQLQPFPQPQLPYPQPQLPYPQPQLPYPQPQPFRPQQPYPQSQPQYSQPQQPISQQQQQQQQQQQQKQQQQQQQQILQQILQQQLIPCRDVVLQQHSIAYGSSQVLQQSTYQLVQQLCCQQLWQIPEQSRCQAIHNVVHAIILHQQQQQQQQQQQQPLSQVSFQQPQQQYPSGQGSFQPSQQNPQAQGSVQPQQLPQFEEIRNLALETLPAMCNVYIPPYCTIAPVGIFGTNYR

SEQ ID NO: 8 - protein, 269 aa, Triticum aestivum
MVRVPVPQLQPQNPSQQQPQEQVPLVQQQQFLGQQQPFPPQQPYPQPQPFPSQLPYLQLQPFPQPQLPYSQPQPFRPQQPYPQPQPQYSQPQQPISQQQQQQQQQQQQQQQQQQILQQILQQQLIPCMDVVLQQHNIAHGRSQVLQQSTYQLLQELCCQHLWQIPEQSQCQAIHNVVHAIILHQQQKQQQQPSSQVSFQQPLQQYPLGQGSFRPSQQNPQAQGSVQPQQLPQFEEIRNLALQTLPAMCNVYIPPYCTIAPFGIFGTNYR

SEQ ID NO: 9 - protein, 210 aa, Triticum aestivum
MKTFLILALLAIVATTATTAVRVPVPQYSQPQQPISQQQQQQQQQQQQQILQQILQQQLIPCRDVVLQQHNIAHGSSQVLQESTYQLVQQLCCQQLWQIPEQSRCQAIHNVVHAIILHQQHHHHQQQQQQQQQQPLSQVSFQQPQQQYPSGQGFFQPSQQNPQAQGSFQPQQLPQFEAIRNLALQTLPAMCNVYIPPYCTIAPFGIFGTN

SEQ ID NO: 10 - protein, 313 aa, Triticum turgidum
MKTFLILALLAIVATTATTAVRVPVPQLQPQNPSQQQPQEQVPLVQQQQFPGQQQQFPPQQPYPQPQPFPSQQPYLQLQPFPQPQPFPPQLPYPQPQSFPPQQPYPQQQPQYLQPQQQISQQQAQQQQQQQQQQQQQQQILQQILQQQLIPCRDVVLQQHNIAHASSQVLQQSTYQLLQQLCCQQLLQIPEQSRCQAIHNVAHAIIMHQQQQQQQEQQQQLQQQQQQQLHQQRQQPSSQVSFQQPQQQYPSSQVSFQPSQLNPQAQGSVQPQQLPQFAEIRNLALQTLPAMCNVYIPPHCSTTIAPFGIFGTN